European Patent Application EP 4 722 245 A1, published April 8, 2026. Title: 靶向ITGA2的抗体、其抗体药物缀合物以及用途. Applicant: 昱言科技（北京）有限公司. Application CN. The sequence listing filed with the application follows.

SEQUENCE LISTING (242 sequences)

SEQ ID NO: 1 - DNA, 642 bp, synthetic construct
  source 1..642: mol_type = other DNA
gacatcgtgatgacccagtctccaaagtccatgtccatgagcgtgggcgagagagtgaccctgtcttgcaaggcctctgagaacgtgggcacctacgtgtcctggtatcagcagaagcctgagcagtcccctaagctgctgatctacggcgcctccaccagagaatctggcgtgcccgatagattcaccggctctggctctggcaccgactttaccctgaccatcagctctgtgcaggccgaggatctggccgtgtactactgccagaacgactacagctaccccttcacctttggctccggcaccaagctggaaatcaagaggaccgtggctgcccccagcgtgttcatcttccctcctagcgacgagcagctgaagagcggcaccgctagcgtggtgtgtctgctgaataacttctatcccagggaggccaaggtgcagtggaaggtggataacgccctgcagagcggcaactcccaggagtccgtgaccgagcaggactccaaggacagcacctactccctgagctccaccctgaccctgtccaaggctgattatgagaagcacaaggtgtatgcttgcgaggtgacacaccagggcctgtccagccctgtgaccaagagcttcaaccggggcgagtgc

SEQ ID NO: 2 - DNA, 1362 bp, synthetic construct
  source 1..1362: mol_type = other DNA
caggttcagttgcagcagtctggcgccgaactcgttagacctggcgcttctgtgaccctgtcctgcaaggcttctggctacaccttcaccgactacgagatgcactgggtcaagcagacccctgtgcatggcctggaatggatcggcgtgatcgatcctgagacaggcggcaccacctacaaccagaagttcaacgacaaggctaccctgaccgccgacaagtcctcttccaccgcctacatggacctgcggtccctgacctctgaggactctgccgtgtactactgctccagatccggctactacgtgtcctcctacgagtcctacgctatggactattggggccagggcacctccgtgacagtctcttctgcttccaccaagggcccctccgtgttccccctggctccctcttccaagagcaccagcggcggcaccgctgctctgggatgtctggtgaaggactacttccctgagcctgtgaccgtgtcctggaattccggcgccctgacctccggcgtgcacacattccctgctgtgctgcagtcctccggcctgtatagcctgtcctccgtggtgacagtgcctagctccagcctgggcacccagacctatatctgcaacgtgaaccacaagcctagcaataccaaggtggacaagaaggtggagcctaagagctgcgacaagacccacacctgtcctccatgtcctgctccagaactgctcggcggaccttccgtgttcctgtttcctccaaagcctaaggacaccctgatgatcagcagaacccctgaagtgacctgcgtggtggtggatgtgtcccacgaggatcccgaagtgaagttcaattggtacgtggacggcgtggaagtgcacaacgccaagaccaagcctagagaggaacagtacaacagcacctacagagtggtgtccgtgctgaccgtgctgcaccaggattggctgaacggcaaagagtacaagtgcaaggtgtccaacaaggccctgcctgctcctatcgagaaaaccatcagcaaggccaagggccagcctagggaaccccaggtttacacactgcctccaagcagggacgagctgaccaagaatcaggtgtccctgacctgcctggtcaagggcttctacccttccgatatcgccgtggaatgggagagcaatggccagcctgagaacaactacaagacaacccctcctgtgctggacagcgacggctcattcttcctgtacagcaagctgacagtggacaagagcagatggcagcagggcaacgtgttcagctgcagcgtgatgcacgaggccctgcacaaccactacacccagaagtccctgagcctgtctcctggcaaa

SEQ ID NO: 3 - DNA, 642 bp, synthetic construct
  source 1..642: mol_type = other DNA
gagatcgtgatgacccagtctcctaagaccatgtccatgtctcccggcgagagagtgaccctgtcttgcaaggcctctgagaacgtgggcacctacgtgtcctggtatcagcagaagcctggacaggcccctcggctgttgatctacggcgcttccacaagagaatccggcgtgcccgatagattctccggctctggctctggcaccgactttaccctgacaatctccagcctgcagcctgaggacttcgccgtgtactactgccagaacgactacagctaccccttcacctttggcggaggcaccaagctggaaatcaagaggaccgtggctgcccccagcgtgttcatcttccctcctagcgacgagcagctgaagagcggcaccgctagcgtggtgtgtctgctgaataacttctatcccagggaggccaaggtgcagtggaaggtggataacgccctgcagagcggcaactcccaggagtccgtgaccgagcaggactccaaggacagcacctactccctgagctccaccctgaccctgtccaaggctgattatgagaagcacaaggtgtatgcttgcgaggtgacacaccagggcctgtccagccctgtgaccaagagcttcaaccggggcgagtgc

SEQ ID NO: 4 - DNA, 1362 bp, synthetic construct
  source 1..1362: mol_type = other DNA
caggttcagctggttcagtctggcgccgaagtgaagaaacctggcgcctctgtgaaggtgtcctgcaaggcttctggctacacctttaccgactacgagatgcactgggtccgacaggctccaggacaaggcttggaatggatgggcgtgatcgaccctgagacaggcggcaccacctacaaccagaaattccagggcagagtgaccctgaccgccgacacctctatctccaccgcctacatggaactgtcccggctgagatctgacgacaccgccgtgtactactgctccagatccggctactacgtgtcctcctacgagtcctacgctatggactattggggccagggcaccaccgtgacagtctcttctgcttccaccaagggcccctccgtgttccccctggctccctcttccaagagcaccagcggcggcaccgctgctctgggatgtctggtgaaggactacttccctgagcctgtgaccgtgtcctggaattccggcgccctgacctccggcgtgcacacattccctgctgtgctgcagtcctccggcctgtatagcctgtcctccgtggtgacagtgcctagctccagcctgggcacccagacctatatctgcaacgtgaaccacaagcctagcaataccaaggtggacaagaaggtggagcctaagagctgcgacaagacccacacctgtcctccatgtcctgctccagaactgctcggcggaccttccgtgttcctgtttcctccaaagcctaaggacaccctgatgatcagcagaacccctgaagtgacctgcgtggtggtggatgtgtcccacgaggatcccgaagtgaagttcaattggtacgtggacggcgtggaagtgcacaacgccaagaccaagcctagagaggaacagtacaacagcacctacagagtggtgtccgtgctgaccgtgctgcaccaggattggctgaacggcaaagagtacaagtgcaaggtgtccaacaaggccctgcctgctcctatcgagaaaaccatcagcaaggccaagggccagcctagggaaccccaggtttacacactgcctccaagcagggacgagctgaccaagaatcaggtgtccctgacctgcctggtcaagggcttctacccttccgatatcgccgtggaatgggagagcaatggccagcctgagaacaactacaagacaacccctcctgtgctggacagcgacggctcattcttcctgtacagcaagctgacagtggacaagagcagatggcagcagggcaacgtgttcagctgcagcgtgatgcacgaggccctgcacaaccactacacccagaagtccctgagcctgtctcctggcaaa

SEQ ID NO: 5 - DNA, 642 bp, synthetic construct
  source 1..642: mol_type = other DNA
gagatcgtgatgacccagtctcctcctaccatgtccatgtctcccggcgagagagtgaccctgtcttgcaaggcctctgagaacgtgggcacctacgtgtcctggtatcagcagaagcctggacaggcccctcggctgttgatctacggcgcttccacaagagaatccggcgtgccagccagattctccggctctggatctggcaccgactttaccctgacaatctccagcctgcagcctgaggacttcgccgtgtactactgccagaacgactacagctaccccttcacctttggcggaggcaccaagctggaaatcaagaggaccgtggctgcccccagcgtgttcatcttccctcctagcgacgagcagctgaagagcggcaccgctagcgtggtgtgtctgctgaataacttctatcccagggaggccaaggtgcagtggaaggtggataacgccctgcagagcggcaactcccaggagtccgtgaccgagcaggactccaaggacagcacctactccctgagctccaccctgaccctgtccaaggctgattatgagaagcacaaggtgtatgcttgcgaggtgacacaccagggcctgtccagccctgtgaccaagagcttcaaccggggcgagtgc

SEQ ID NO: 6 - DNA, 1362 bp, synthetic construct; identical to SEQ ID NO: 4
  source 1..1362: mol_type = other DNA

SEQ ID NO: 7 - DNA, 642 bp, synthetic construct
  source 1..642: mol_type = other DNA
gagatcgtgatgacccagtctcctcctacactgtctctgagccctggcgagagagtgaccctgtcttgtagagcctctgagaacgtgggcacctacgtgtcctggtatcagcagaagcctggacaggcccctcggctgttgatctacggcgcttctaccagagagagcggcatccctgccagattctccggctctggctctggcacagactttaccctgacaatctccagcctgcagcctgaggacttcgccgtgtactactgccagaacgactacagctaccccttcacctttggcggaggcaccaagctggaaatcaagaggaccgtggctgcccccagcgtgttcatcttccctcctagcgacgagcagctgaagagcggcaccgctagcgtggtgtgtctgctgaataacttctatcccagggaggccaaggtgcagtggaaggtggataacgccctgcagagcggcaactcccaggagtccgtgaccgagcaggactccaaggacagcacctactccctgagctccaccctgaccctgtccaaggctgattatgagaagcacaaggtgtatgcttgcgaggtgacacaccagggcctgtccagccctgtgaccaagagcttcaaccggggcgagtgc

SEQ ID NO: 8 - DNA, 1362 bp, synthetic construct; identical to SEQ ID NO: 4
  source 1..1362: mol_type = other DNA

SEQ ID NO: 9 - DNA, 660 bp, synthetic construct
  source 1..660: mol_type = other DNA
gacatcgtgatgacccagtctccatccagcctgaccgtgaccgctggcgagaaagtgaccatgtcctgcaagtcctctcagtccctgctgaactccggcaaccagaagaactacctgacctggtatcagcagaagcccggccagcctcctaagctgttgatctacggcgcctccaccagagaatctggcgtgcccgatagattcaccggctctggctctggcaccgactttaccctgaccatcagctctgtgcaggccgaggatctggccgtgtactactgccagaacgactacagctaccccttcacctttggctccggcaccaagctggaaatcaagaggaccgtggctgcccccagcgtgttcatcttccctcctagcgacgagcagctgaagagcggcaccgctagcgtggtgtgtctgctgaataacttctatcccagggaggccaaggtgcagtggaaggtggataacgccctgcagagcggcaactcccaggagtccgtgaccgagcaggactccaaggacagcacctactccctgagctccaccctgaccctgtccaaggctgattatgagaagcacaaggtgtatgcttgcgaggtgacacaccagggcctgtccagccctgtgaccaagagcttcaaccggggcgagtgc

SEQ ID NO: 10 - DNA, 1362 bp, synthetic construct
  source 1..1362: mol_type = other DNA
caggttcagttgcagcagtctggcgccgaactcgttagacctggcgcttctgtgaccctgtcctgcaaggcttctggctacaccttcaccgactacgagatgcactgggtcaagcagacccctgtgcatggcctggaatggatcggcaccatcgatcctgagacaggcggcaccacctacaaccagaagttcaacgacaaggctaccctgaccgccgacaagtcctcttccaccgcctacatggacctgcggtccctgacctctgaggactctgccgtgtactactgctccagatccggctactacgtgtcctcctacgagtcctacgctatggactattggggccagggcacctccgtgacagtctcttctgcttccaccaagggcccctccgtgttccccctggctccctcttccaagagcaccagcggcggcaccgctgctctgggatgtctggtgaaggactacttccctgagcctgtgaccgtgtcctggaattccggcgccctgacctccggcgtgcacacattccctgctgtgctgcagtcctccggcctgtatagcctgtcctccgtggtgacagtgcctagctccagcctgggcacccagacctatatctgcaacgtgaaccacaagcctagcaataccaaggtggacaagaaggtggagcctaagagctgcgacaagacccacacctgtcctccatgtcctgctccagaactgctcggcggaccttccgtgttcctgtttcctccaaagcctaaggacaccctgatgatcagcagaacccctgaagtgacctgcgtggtggtggatgtgtcccacgaggatcccgaagtgaagttcaattggtacgtggacggcgtggaagtgcacaacgccaagaccaagcctagagaggaacagtacaacagcacctacagagtggtgtccgtgctgaccgtgctgcaccaggattggctgaacggcaaagagtacaagtgcaaggtgtccaacaaggccctgcctgctcctatcgagaaaaccatcagcaaggccaagggccagcctagggaaccccaggtttacacactgcctccaagcagggacgagctgaccaagaatcaggtgtccctgacctgcctggtcaagggcttctacccttccgatatcgccgtggaatgggagagcaatggccagcctgagaacaactacaagacaacccctcctgtgctggacagcgacggctcattcttcctgtacagcaagctgacagtggacaagagcagatggcagcagggcaacgtgttcagctgcagcgtgatgcacgaggccctgcacaaccactacacccagaagtccctgagcctgtctcctggcaaa

SEQ ID NO: 11 - DNA, 660 bp, synthetic construct
  source 1..660: mol_type = other DNA
gacatcgtgatgacccagtctccagacagcctggctgtgtctctgggcgagagagccaccatcaactgcaagtcctctcagtccctgctgaactccggcaaccagaagaactacctgacctggtatcagcagaagcccggccagcctcctaagctgttgatctacggcgcctccaccagagaatctggcgtgcccgatagattctccggctctggctctggcaccgactttaccctgacaatcagctccctgcaggccgaggatgtggccgtgtactactgccagaacgactacagctaccccttcacctttggcggaggcaccaagctggaaatcaagaggaccgtggctgcccccagcgtgttcatcttccctcctagcgacgagcagctgaagagcggcaccgctagcgtggtgtgtctgctgaataacttctatcccagggaggccaaggtgcagtggaaggtggataacgccctgcagagcggcaactcccaggagtccgtgaccgagcaggactccaaggacagcacctactccctgagctccaccctgaccctgtccaaggctgattatgagaagcacaaggtgtatgcttgcgaggtgacacaccagggcctgtccagccctgtgaccaagagcttcaaccggggcgagtgc

SEQ ID NO: 12 - DNA, 1362 bp, synthetic construct
  source 1..1362: mol_type = other DNA
caggttcagctggttcagtctggcgccgaagtgaagaaacctggcgcctccgtgaagctgtcctgcaaggcttctggctacaccttcaccgactacgagatgcactgggtccgacaggctccaggacaaggcctggaatggatcggcaccatcgatcctgagacaggcggcaccacctacaaccagaaattccagggcagagtgaccctgaccgccgacacctctatctccaccgcctacatggaactgtcccggctgagatctgacgacaccgccgtgtactactgctccagatccggctactacgtgtcctcctacgagtcctacgctatggactattggggccagggcaccaccgtgacagtctcttctgcttccaccaagggcccctccgtgttccccctggctccctcttccaagagcaccagcggcggcaccgctgctctgggatgtctggtgaaggactacttccctgagcctgtgaccgtgtcctggaattccggcgccctgacctccggcgtgcacacattccctgctgtgctgcagtcctccggcctgtatagcctgtcctccgtggtgacagtgcctagctccagcctgggcacccagacctatatctgcaacgtgaaccacaagcctagcaataccaaggtggacaagaaggtggagcctaagagctgcgacaagacccacacctgtcctccatgtcctgctccagaactgctcggcggaccttccgtgttcctgtttcctccaaagcctaaggacaccctgatgatcagcagaacccctgaagtgacctgcgtggtggtggatgtgtcccacgaggatcccgaagtgaagttcaattggtacgtggacggcgtggaagtgcacaacgccaagaccaagcctagagaggaacagtacaacagcacctacagagtggtgtccgtgctgaccgtgctgcaccaggattggctgaacggcaaagagtacaagtgcaaggtgtccaacaaggccctgcctgctcctatcgagaaaaccatcagcaaggccaagggccagcctagggaaccccaggtttacacactgcctccaagcagggacgagctgaccaagaatcaggtgtccctgacctgcctggtcaagggcttctacccttccgatatcgccgtggaatgggagagcaatggccagcctgagaacaactacaagacaacccctcctgtgctggacagcgacggctcattcttcctgtacagcaagctgacagtggacaagagcagatggcagcagggcaacgtgttcagctgcagcgtgatgcacgaggccctgcacaaccactacacccagaagtccctgagcctgtctcctggcaaa

SEQ ID NO: 13 - DNA, 660 bp, synthetic construct
  source 1..660: mol_type = other DNA
gacatcgtgatgacccagtctccagacagcctggctgtgtctctgggcgagcgcgtgaccatgaactgcaagtcctctcagtccctgctgaactccggcaaccagaagaactacctgacctggtatcagcagaagcccggccagcctcctaagctgttgatctacggcgcctccaccagagaatctggcgtgcccgatagattctccggctctggctctggcaccgactttaccctgacaatcagctccctgcaggccgaggatgtggccgtgtactactgccagaacgactacagctaccccttcacctttggcggaggcaccaagctggaaatcaagaggaccgtggctgcccccagcgtgttcatcttccctcctagcgacgagcagctgaagagcggcaccgctagcgtggtgtgtctgctgaataacttctatcccagggaggccaaggtgcagtggaaggtggataacgccctgcagagcggcaactcccaggagtccgtgaccgagcaggactccaaggacagcacctactccctgagctccaccctgaccctgtccaaggctgattatgagaagcacaaggtgtatgcttgcgaggtgacacaccagggcctgtccagccctgtgaccaagagcttcaaccggggcgagtgc

SEQ ID NO: 14 - DNA, 1362 bp, synthetic construct
  source 1..1362: mol_type = other DNA
caggttcagctggttcagtctggcgccgaagtgaagaaacctggcgcctctgtgaaggtgtcctgcaaggcttctggctacacctttaccgactacgagatgcactgggtccgacaggctccaggacaaggcttggagtggatgggcaccatcgatcctgagacaggcggcaccacctacgctcagaaattccagggcagagtgaccctgaccgccgacacctctatctccaccgcctacatggaactgtcccggctgagatctgacgacaccgccgtgtactactgctccagatccggctactacgtgtcctcctacgagtcctacgctatggactattggggccagggcaccaccgtgacagtctcttctgcttccaccaagggcccctccgtgttccccctggctccctcttccaagagcaccagcggcggcaccgctgctctgggatgtctggtgaaggactacttccctgagcctgtgaccgtgtcctggaattccggcgccctgacctccggcgtgcacacattccctgctgtgctgcagtcctccggcctgtatagcctgtcctccgtggtgacagtgcctagctccagcctgggcacccagacctatatctgcaacgtgaaccacaagcctagcaataccaaggtggacaagaaggtggagcctaagagctgcgacaagacccacacctgtcctccatgtcctgctccagaactgctcggcggaccttccgtgttcctgtttcctccaaagcctaaggacaccctgatgatcagcagaacccctgaagtgacctgcgtggtggtggatgtgtcccacgaggatcccgaagtgaagttcaattggtacgtggacggcgtggaagtgcacaacgccaagaccaagcctagagaggaacagtacaacagcacctacagagtggtgtccgtgctgaccgtgctgcaccaggattggctgaacggcaaagagtacaagtgcaaggtgtccaacaaggccctgcctgctcctatcgagaaaaccatcagcaaggccaagggccagcctagggaaccccaggtttacacactgcctccaagcagggacgagctgaccaagaatcaggtgtccctgacctgcctggtcaagggcttctacccttccgatatcgccgtggaatgggagagcaatggccagcctgagaacaactacaagacaacccctcctgtgctggacagcgacggctcattcttcctgtacagcaagctgacagtggacaagagcagatggcagcagggcaacgtgttcagctgcagcgtgatgcacgaggccctgcacaaccactacacccagaagtccctgagcctgtctcctggcaaa

SEQ ID NO: 15 - DNA, 660 bp, synthetic construct
  source 1..660: mol_type = other DNA
gacatcgtgatgacccagtctccagacagcctggctgtgtctctgggcgagcgagtgaccatgtcctgcaagtcctctcagtccctgctgaactccggcaaccagaagaactacctgacctggtatcagcagaagcccggccagcctcctaagctgttgatctacggcgcctccaccagagaatctggcgtgcccgatagattcaccggctctggctctggcaccgactttaccctgacaatcagctccctgcaggccgaggatgtggccgtgtactactgccagaacgactacagctaccccttcacctttggcggaggcaccaagctggaaatcaagaggaccgtggctgcccccagcgtgttcatcttccctcctagcgacgagcagctgaagagcggcaccgctagcgtggtgtgtctgctgaataacttctatcccagggaggccaaggtgcagtggaaggtggataacgccctgcagagcggcaactcccaggagtccgtgaccgagcaggactccaaggacagcacctactccctgagctccaccctgaccctgtccaaggctgattatgagaagcacaaggtgtatgcttgcgaggtgacacaccagggcctgtccagccctgtgaccaagagcttcaaccggggcgagtgc

SEQ ID NO: 16 - DNA, 1362 bp, synthetic construct
  source 1..1362: mol_type = other DNA
caggttcagctggttcagtctggcgccgaagtgaagaaacctggcgcctctgtgaaggtgtcctgcaaggcttctggctacacctttaccgactacgagatgcactgggtccgacaggctccaggacaaggcttggagtggatgggcaccatcgatcctgagacaggcggcaccacctacgctcagaaattccagggcagagtgaccatgaccgccgacacctctatctccaccgcctacatggaactgtcccggctgagatctgacgacaccgccgtgtactactgtgccagatccggctactacgtgtcctcctacgagtcctacgctatggactattggggccagggcaccaccgtgacagtctcttctgcttccaccaagggcccctccgtgttccccctggctccctcttccaagagcaccagcggcggcaccgctgctctgggatgtctggtgaaggactacttccctgagcctgtgaccgtgtcctggaattccggcgccctgacctccggcgtgcacacattccctgctgtgctgcagtcctccggcctgtatagcctgtcctccgtggtgacagtgcctagctccagcctgggcacccagacctatatctgcaacgtgaaccacaagcctagcaataccaaggtggacaagaaggtggagcctaagagctgcgacaagacccacacctgtcctccatgtcctgctccagaactgctcggcggaccttccgtgttcctgtttcctccaaagcctaaggacaccctgatgatcagcagaacccctgaagtgacctgcgtggtggtggatgtgtcccacgaggatcccgaagtgaagttcaattggtacgtggacggcgtggaagtgcacaacgccaagaccaagcctagagaggaacagtacaacagcacctacagagtggtgtccgtgctgaccgtgctgcaccaggattggctgaacggcaaagagtacaagtgcaaggtgtccaacaaggccctgcctgctcctatcgagaaaaccatcagcaaggccaagggccagcctagggaaccccaggtttacacactgcctccaagcagggacgagctgaccaagaatcaggtgtccctgacctgcctggtcaagggcttctacccttccgatatcgccgtggaatgggagagcaatggccagcctgagaacaactacaagacaacccctcctgtgctggacagcgacggctcattcttcctgtacagcaagctgacagtggacaagagcagatggcagcagggcaacgtgttcagctgcagcgtgatgcacgaggccctgcacaaccactacacccagaagtccctgagcctgtctcctggcaaa

SEQ ID NO: 17 - DNA, 660 bp, synthetic construct; identical to SEQ ID NO: 13
  source 1..660: mol_type = other DNA

SEQ ID NO: 18 - DNA, 1362 bp, synthetic construct; identical to SEQ ID NO: 16
  source 1..1362: mol_type = other DNA

SEQ ID NO: 19 - DNA, 660 bp, synthetic construct
  source 1..660: mol_type = other DNA
gacatcgtgatgacccagtctccacctacactgtccgtgtctccaggcgagcgcgtgaccatgtcttgcaagtcctctcagtccctgctgaactccggcaaccagaagaactacctgacctggtatcagcagaagcccggccaggctcctagactgttgatctacggcgcctccaccagagaatctggcgtgcccgatagattctccggctctggctctggcaccgactttaccctgacaatctccagcctgcagcctgaggacttcgccgtgtactactgccagaacgactacagctaccccttcacctttggcggaggcaccaagctggaaatcaagaggaccgtggctgcccccagcgtgttcatcttccctcctagcgacgagcagctgaagagcggcaccgctagcgtggtgtgtctgctgaataacttctatcccagggaggccaaggtgcagtggaaggtggataacgccctgcagagcggcaactcccaggagtccgtgaccgagcaggactccaaggacagcacctactccctgagctccaccctgaccctgtccaaggctgattatgagaagcacaaggtgtatgcttgcgaggtgacacaccagggcctgtccagccctgtgaccaagagcttcaaccggggcgagtgc

SEQ ID NO: 20 - DNA, 1362 bp, synthetic construct; identical to SEQ ID NO: 16
  source 1..1362: mol_type = other DNA

SEQ ID NO: 21 - DNA, 660 bp, synthetic construct
  source 1..660: mol_type = other DNA
gagatcgtgatgacccagtctcctcctacactgtctctgagccctggcgagcgcgtgaccatgtcctgtagatcctctcagtccctgctgaactccggcaaccagaagaactacctgacctggtatcagcagaagcccggccaggctcctagactgttgatctacggcgcctccaccagagaatctggcgtgccagctagattctccggctctggctctggcaccgactttaccctgacaatctccagcctgcagcctgaggacttcgccgtgtactactgccagaacgactacagctaccccttcacctttggcggaggcaccaagctggaaatcaagaggaccgtggctgcccccagcgtgttcatcttccctcctagcgacgagcagctgaagagcggcaccgctagcgtggtgtgtctgctgaataacttctatcccagggaggccaaggtgcagtggaaggtggataacgccctgcagagcggcaactcccaggagtccgtgaccgagcaggactccaaggacagcacctactccctgagctccaccctgaccctgtccaaggctgattatgagaagcacaaggtgtatgcttgcgaggtgacacaccagggcctgtccagccctgtgaccaagagcttcaaccggggcgagtgc

SEQ ID NO: 22 - DNA, 1362 bp, synthetic construct; identical to SEQ ID NO: 16
  source 1..1362: mol_type = other DNA

SEQ ID NO: 23 - DNA, 642 bp, synthetic construct
  source 1..642: mol_type = other DNA
gacatcgtgatgacccagagccagaaattcatgtccacctccgtgggcgacagagtgtccgtgacatgcaaggcctctcagaacgtgggcaccaacgtggcctggtatcagcagaagcctggccagtctcctaagactctgatctactccgcctcctaccggttctctggcgtgcccgatagattcaccggctctggatctggcaccgacttcaccctgaccatcaacaacgtgcagtccgaggacctggccgactacttctgccagcagtacaacatctaccctctgtccttcggcgctggcaccaagctggaactgaaaaggaccgtggctgcccccagcgtgttcatcttccctcctagcgacgagcagctgaagagcggcaccgctagcgtggtgtgtctgctgaataacttctatcccagggaggccaaggtgcagtggaaggtggataacgccctgcagagcggcaactcccaggagtccgtgaccgagcaggactccaaggacagcacctactccctgagctccaccctgaccctgtccaaggctgattatgagaagcacaaggtgtatgcttgcgaggtgacacaccagggcctgtccagccctgtgaccaagagcttcaaccggggcgagtgc

SEQ ID NO: 24 - DNA, 1362 bp, synthetic construct
  source 1..1362: mol_type = other DNA
caggttcagttgcagcagtctggcgccgaactcgttagacctggcgcttctgtgaccctgtcctgcaaggcttctggctacaccttcaccgactacgagatccactgggtcaagcagacccctgtgcatggcctggaatggatcggcgccatcgatcctgaaaccggcggcaccaactacaaccagaagttcaacgacaaggctaccctgaccgccgacaagtcctcttccaccgcctacatggacctgcggtccctgacctctgaggactctgccgtgtactactgctccagatccggctactacgtgtccaactacgagtcctacgctatggactactggggccagggcacctctgtgacagtctcttctgcttccaccaagggcccctccgtgttccccctggctccctcttccaagagcaccagcggcggcaccgctgctctgggatgtctggtgaaggactacttccctgagcctgtgaccgtgtcctggaattccggcgccctgacctccggcgtgcacacattccctgctgtgctgcagtcctccggcctgtatagcctgtcctccgtggtgacagtgcctagctccagcctgggcacccagacctatatctgcaacgtgaaccacaagcctagcaataccaaggtggacaagaaggtggagcctaagagctgcgacaagacccacacctgtcctccatgtcctgctccagaactgctcggcggaccttccgtgttcctgtttcctccaaagcctaaggacaccctgatgatcagcagaacccctgaagtgacctgcgtggtggtggatgtgtcccacgaggatcccgaagtgaagttcaattggtacgtggacggcgtggaagtgcacaacgccaagaccaagcctagagaggaacagtacaacagcacctacagagtggtgtccgtgctgaccgtgctgcaccaggattggctgaacggcaaagagtacaagtgcaaggtgtccaacaaggccctgcctgctcctatcgagaaaaccatcagcaaggccaagggccagcctagggaaccccaggtttacacactgcctccaagcagggacgagctgaccaagaatcaggtgtccctgacctgcctggtcaagggcttctacccttccgatatcgccgtggaatgggagagcaatggccagcctgagaacaactacaagacaacccctcctgtgctggacagcgacggctcattcttcctgtacagcaagctgacagtggacaagagcagatggcagcagggcaacgtgttcagctgcagcgtgatgcacgaggccctgcacaaccactacacccagaagtccctgagcctgtctcctggcaaa

SEQ ID NO: 25 - DNA, 642 bp, synthetic construct
  source 1..642: mol_type = other DNA
gacatccagatgacccagtctccatcctctctgtccgcctctgtgggcgacagagtgaccatcacctgtcgggcctctcagaacgtgggcaccaatgtggcttggtatcagcagaagcccgagaaggcccctaagagcctgatctactccgcctcctaccggttctctggcgtgccctctagattctccggctctggctctggcaccgactttaccctgacaatctccagcctgcagcctgaggacttcgccacctactactgccagcagtacaacatctaccctctgtccttcggcggaggcaccaagctggaactgaaaaggaccgtggctgcccccagcgtgttcatcttccctcctagcgacgagcagctgaagagcggcaccgctagcgtggtgtgtctgctgaataacttctatcccagggaggccaaggtgcagtggaaggtggataacgccctgcagagcggcaactcccaggagtccgtgaccgagcaggactccaaggacagcacctactccctgagctccaccctgaccctgtccaaggctgattatgagaagcacaaggtgtatgcttgcgaggtgacacaccagggcctgtccagccctgtgaccaagagcttcaaccggggcgagtgc

SEQ ID NO: 26 - DNA, 1362 bp, synthetic construct
  source 1..1362: mol_type = other DNA
caggttcagctggttcagtctggcgccgaagtgaagaaacctggcgcctctgtgaaggtgtcctgcaaggcttctggctacacctttaccgactacgagatccactgggtccgacaggctccaggacaaggcctggaatggatcggcgccatcgatcctgaaaccggcggcaccaactacaaccagaaattcaacgacagagtgaccctgaccgccgacaagtccatctccaccgcctacatggaactgtcccggctgagatctgacgacaccgccgtgtactactgctccagatccggctactacgtgtccaactacgagtcctacgctatggactactggggccagggcaccacagtgacagtctcttctgcttccaccaagggcccctccgtgttccccctggctccctcttccaagagcaccagcggcggcaccgctgctctgggatgtctggtgaaggactacttccctgagcctgtgaccgtgtcctggaattccggcgccctgacctccggcgtgcacacattccctgctgtgctgcagtcctccggcctgtatagcctgtcctccgtggtgacagtgcctagctccagcctgggcacccagacctatatctgcaacgtgaaccacaagcctagcaataccaaggtggacaagaaggtggagcctaagagctgcgacaagacccacacctgtcctccatgtcctgctccagaactgctcggcggaccttccgtgttcctgtttcctccaaagcctaaggacaccctgatgatcagcagaacccctgaagtgacctgcgtggtggtggatgtgtcccacgaggatcccgaagtgaagttcaattggtacgtggacggcgtggaagtgcacaacgccaagaccaagcctagagaggaacagtacaacagcacctacagagtggtgtccgtgctgaccgtgctgcaccaggattggctgaacggcaaagagtacaagtgcaaggtgtccaacaaggccctgcctgctcctatcgagaaaaccatcagcaaggccaagggccagcctagggaaccccaggtttacacactgcctccaagcagggacgagctgaccaagaatcaggtgtccctgacctgcctggtcaagggcttctacccttccgatatcgccgtggaatgggagagcaatggccagcctgagaacaactacaagacaacccctcctgtgctggacagcgacggctcattcttcctgtacagcaagctgacagtggacaagagcagatggcagcagggcaacgtgttcagctgcagcgtgatgcacgaggccctgcacaaccactacacccagaagtccctgagcctgtctcctggcaaa

SEQ ID NO: 27 - DNA, 642 bp, synthetic construct; identical to SEQ ID NO: 25
  source 1..642: mol_type = other DNA

SEQ ID NO: 28 - DNA, 1362 bp, synthetic construct
  source 1..1362: mol_type = other DNA
caggttcagctggttcagtctggcgccgaagtgaagaaacctggcgcctctgtgaaggtgtcctgcaaggcttctggctacacctttaccgactacgagatccactgggtccgacaggctccaggacaaggcctggaatggatcggcgccatcgatcctgaaaccggcggcaccaactacaaccagaaattccagggcagagtgaccctgaccgccgacacctctatctccaccgcctacatggaactgtcccggctgagatctgacgacaccgccgtgtactactgctccagatccggctactacgtgtccaactacgagtcctacgctatggactactggggccagggcaccacagtgacagtctcttctgcttccaccaagggcccctccgtgttccccctggctccctcttccaagagcaccagcggcggcaccgctgctctgggatgtctggtgaaggactacttccctgagcctgtgaccgtgtcctggaattccggcgccctgacctccggcgtgcacacattccctgctgtgctgcagtcctccggcctgtatagcctgtcctccgtggtgacagtgcctagctccagcctgggcacccagacctatatctgcaacgtgaaccacaagcctagcaataccaaggtggacaagaaggtggagcctaagagctgcgacaagacccacacctgtcctccatgtcctgctccagaactgctcggcggaccttccgtgttcctgtttcctccaaagcctaaggacaccctgatgatcagcagaacccctgaagtgacctgcgtggtggtggatgtgtcccacgaggatcccgaagtgaagttcaattggtacgtggacggcgtggaagtgcacaacgccaagaccaagcctagagaggaacagtacaacagcacctacagagtggtgtccgtgctgaccgtgctgcaccaggattggctgaacggcaaagagtacaagtgcaaggtgtccaacaaggccctgcctgctcctatcgagaaaaccatcagcaaggccaagggccagcctagggaaccccaggtttacacactgcctccaagcagggacgagctgaccaagaatcaggtgtccctgacctgcctggtcaagggcttctacccttccgatatcgccgtggaatgggagagcaatggccagcctgagaacaactacaagacaacccctcctgtgctggacagcgacggctcattcttcctgtacagcaagctgacagtggacaagagcagatggcagcagggcaacgtgttcagctgcagcgtgatgcacgaggccctgcacaaccactacacccagaagtccctgagcctgtctcctggcaaa

SEQ ID NO: 29 - DNA, 642 bp, synthetic construct; identical to SEQ ID NO: 25
  source 1..642: mol_type = other DNA

SEQ ID NO: 30 - DNA, 1362 bp, synthetic construct
  source 1..1362: mol_type = other DNA
caggttcagctggttcagtctggcgccgaagtgaagaaacctggcgcctctgtgaaggtgtcctgcaaggcttctggctacacctttaccgactacgagatccactgggtccgacaggctccaggacaaggcttggaatggatgggcgccatcgatcctgagacaggcggcaccaattacgcccagaaattccagggcagagtgaccatgaccgccgacacctctatctccaccgcctacatggaactgtcccggctgagatctgacgacaccgccgtgtactactgctccagatccggctactacgtgtccaactacgagtcctacgctatggactactggggccagggcaccacagtgacagtctcttctgcttccaccaagggcccctccgtgttccccctggctccctcttccaagagcaccagcggcggcaccgctgctctgggatgtctggtgaaggactacttccctgagcctgtgaccgtgtcctggaattccggcgccctgacctccggcgtgcacacattccctgctgtgctgcagtcctccggcctgtatagcctgtcctccgtggtgacagtgcctagctccagcctgggcacccagacctatatctgcaacgtgaaccacaagcctagcaataccaaggtggacaagaaggtggagcctaagagctgcgacaagacccacacctgtcctccatgtcctgctccagaactgctcggcggaccttccgtgttcctgtttcctccaaagcctaaggacaccctgatgatcagcagaacccctgaagtgacctgcgtggtggtggatgtgtcccacgaggatcccgaagtgaagttcaattggtacgtggacggcgtggaagtgcacaacgccaagaccaagcctagagaggaacagtacaacagcacctacagagtggtgtccgtgctgaccgtgctgcaccaggattggctgaacggcaaagagtacaagtgcaaggtgtccaacaaggccctgcctgctcctatcgagaaaaccatcagcaaggccaagggccagcctagggaaccccaggtttacacactgcctccaagcagggacgagctgaccaagaatcaggtgtccctgacctgcctggtcaagggcttctacccttccgatatcgccgtggaatgggagagcaatggccagcctgagaacaactacaagacaacccctcctgtgctggacagcgacggctcattcttcctgtacagcaagctgacagtggacaagagcagatggcagcagggcaacgtgttcagctgcagcgtgatgcacgaggccctgcacaaccactacacccagaagtccctgagcctgtctcctggcaaa

SEQ ID NO: 31 - DNA, 642 bp, synthetic construct
  source 1..642: mol_type = other DNA
gacatcaagatcacccagtctccatcctctatgtacgccagcctgggcgagagagtgaccattacctgcaaggccagccaggacatcaagtcctacctgtcctggtatcagcagaagcccggcagctctcccagactgctgatctacgacacctccaacctggcctctggcgtgccagtcagattttccggcagaggctctggcacctcctacagcctgaccatctccagaatggaagccgaggatgccgccacctactactgtcagcagtggtctagctaccccttcacctttggctccggcaccaagctggaaatcaagaggaccgtggctgcccccagcgtgttcatcttccctcctagcgacgagcagctgaagagcggcaccgctagcgtggtgtgtctgctgaataacttctatcccagggaggccaaggtgcagtggaaggtggataacgccctgcagagcggcaactcccaggagtccgtgaccgagcaggactccaaggacagcacctactccctgagctccaccctgaccctgtccaaggctgattatgagaagcacaaggtgtatgcttgcgaggtgacacaccagggcctgtccagccctgtgaccaagagcttcaaccggggcgagtgc

SEQ ID NO: 32 - DNA, 1362 bp, synthetic construct
  source 1..1362: mol_type = other DNA
cagttgcagttgcagcagtctggcgccgaactcgttagacctggcgcttctgtgaccctgtcctgcaaggcttctggctacaccttcaccgactacgagatccactgggtcaagcagacccctgtgcatggcctggaatggatcggcgccatcgatcctgaaaccggcggcaccaactacaaccagaagttcaacgacaaggctaccctgaccgccgacaagtcctcttccaccgcctacatggacctgcggtccctgacctctgaggactctgccgtgtactactgctccagatccggctactacgtgtccaactacgagtcctacgctatggactactggggccagggcacctctgtgacagtctcttctgcttccaccaagggcccctccgtgttccccctggctccctcttccaagagcaccagcggcggcaccgctgctctgggatgtctggtgaaggactacttccctgagcctgtgaccgtgtcctggaattccggcgccctgacctccggcgtgcacacattccctgctgtgctgcagtcctccggcctgtatagcctgtcctccgtggtgacagtgcctagctccagcctgggcacccagacctatatctgcaacgtgaaccacaagcctagcaataccaaggtggacaagaaggtggagcctaagagctgcgacaagacccacacctgtcctccatgtcctgctccagaactgctcggcggaccttccgtgttcctgtttcctccaaagcctaaggacaccctgatgatcagcagaacccctgaagtgacctgcgtggtggtggatgtgtcccacgaggatcccgaagtgaagttcaattggtacgtggacggcgtggaagtgcacaacgccaagaccaagcctagagaggaacagtacaacagcacctacagagtggtgtccgtgctgaccgtgctgcaccaggattggctgaacggcaaagagtacaagtgcaaggtgtccaacaaggccctgcctgctcctatcgagaaaaccatcagcaaggccaagggccagcctagggaaccccaggtttacacactgcctccaagcagggacgagctgaccaagaatcaggtgtccctgacctgcctggtcaagggcttctacccttccgatatcgccgtggaatgggagagcaatggccagcctgagaacaactacaagacaacccctcctgtgctggacagcgacggctcattcttcctgtacagcaagctgacagtggacaagagcagatggcagcagggcaacgtgttcagctgcagcgtgatgcacgaggccctgcacaaccactacacccagaagtccctgagcctgtctcctggcaaa

SEQ ID NO: 33 - DNA, 642 bp, synthetic construct
  source 1..642: mol_type = other DNA
gacatccagctgacccagtctccatcctctctgtctgcctctgtgggcgacagagtgaccatcacctgtagagccagccaggacatcaagtcctacctgtcctggtatcagcagaagcccggcaaggctcccaagctgctgatctacgacacctccaatctggcctctggcgtgccctctagattctccggttctggctctggcaccgactttaccctgacaatctccagcctgcagcctgaggacttcgccacctactactgtcagcagtggtctagctaccccttcacctttggcggaggcaccaagctggaaatcaagaggaccgtggctgcccccagcgtgttcatcttccctcctagcgacgagcagctgaagagcggcaccgctagcgtggtgtgtctgctgaataacttctatcccagggaggccaaggtgcagtggaaggtggataacgccctgcagagcggcaactcccaggagtccgtgaccgagcaggactccaaggacagcacctactccctgagctccaccctgaccctgtccaaggctgattatgagaagcacaaggtgtatgcttgcgaggtgacacaccagggcctgtccagccctgtgaccaagagcttcaaccggggcgagtgc

SEQ ID NO: 34 - DNA, 1362 bp, synthetic construct
  source 1..1362: mol_type = other DNA
cagctgcagttggttcagtctggcgccgaagtgaagaaacctggcgcctctgtgaaggtgtcctgcaaggcttctggctacacctttaccgactacgagatccactgggtccgacaggctccaggacaaggcctggaatggatcggcgccatcgatcctgaaaccggcggcaccaactacaaccagaaattcaacgacagagtgaccctgaccgccgacacctctatctccaccgcctacatggaactgtcccggctgagatctgacgacaccgccgtgtactactgctccagatccggctactacgtgtccaactacgagtcctacgctatggactactggggccagggcaccacagtgacagtctcttctgcttccaccaagggcccctccgtgttccccctggctccctcttccaagagcaccagcggcggcaccgctgctctgggatgtctggtgaaggactacttccctgagcctgtgaccgtgtcctggaattccggcgccctgacctccggcgtgcacacattccctgctgtgctgcagtcctccggcctgtatagcctgtcctccgtggtgacagtgcctagctccagcctgggcacccagacctatatctgcaacgtgaaccacaagcctagcaataccaaggtggacaagaaggtggagcctaagagctgcgacaagacccacacctgtcctccatgtcctgctccagaactgctcggcggaccttccgtgttcctgtttcctccaaagcctaaggacaccctgatgatcagcagaacccctgaagtgacctgcgtggtggtggatgtgtcccacgaggatcccgaagtgaagttcaattggtacgtggacggcgtggaagtgcacaacgccaagaccaagcctagagaggaacagtacaacagcacctacagagtggtgtccgtgctgaccgtgctgcaccaggattggctgaacggcaaagagtacaagtgcaaggtgtccaacaaggccctgcctgctcctatcgagaaaaccatcagcaaggccaagggccagcctagggaaccccaggtttacacactgcctccaagcagggacgagctgaccaagaatcaggtgtccctgacctgcctggtcaagggcttctacccttccgatatcgccgtggaatgggagagcaatggccagcctgagaacaactacaagacaacccctcctgtgctggacagcgacggctcattcttcctgtacagcaagctgacagtggacaagagcagatggcagcagggcaacgtgttcagctgcagcgtgatgcacgaggccctgcacaaccactacacccagaagtccctgagcctgtctcctggcaaa

SEQ ID NO: 35 - DNA, 642 bp, synthetic construct
  source 1..642: mol_type = other DNA
gacatccagatcacccagtctccatcctccatgtccgcctctgtgggcgacagagtgaccatcacatgcaaggccagccaggacatcaagtcctacctgtcctggtatcagcagaagcccggcaaggctcccaagctgctgatctacgacacctccaatctggcctctggcgtgccctctagattctccggttctggctctggcaccgactataccctgacaatctccagcctgcagcctgaggacttcgccacctactactgtcagcagtggtctagctaccccttcacctttggcggaggcaccaagctggaaatcaagaggaccgtggctgcccccagcgtgttcatcttccctcctagcgacgagcagctgaagagcggcaccgctagcgtggtgtgtctgctgaataacttctatcccagggaggccaaggtgcagtggaaggtggataacgccctgcagagcggcaactcccaggagtccgtgaccgagcaggactccaaggacagcacctactccctgagctccaccctgaccctgtccaaggctgattatgagaagcacaaggtgtatgcttgcgaggtgacacaccagggcctgtccagccctgtgaccaagagcttcaaccggggcgagtgc

SEQ ID NO: 36 - DNA, 1362 bp, synthetic construct; identical to SEQ ID NO: 28
  source 1..1362: mol_type = other DNA

SEQ ID NO: 37 - DNA, 642 bp, synthetic construct; identical to SEQ ID NO: 35
  source 1..642: mol_type = other DNA

SEQ ID NO: 38 - DNA, 1362 bp, synthetic construct; identical to SEQ ID NO: 30
  source 1..1362: mol_type = other DNA

SEQ ID NO: 39 - DNA, 642 bp, synthetic construct; identical to SEQ ID NO: 33
  source 1..642: mol_type = other DNA

SEQ ID NO: 40 - DNA, 1362 bp, synthetic construct; identical to SEQ ID NO: 30
  source 1..1362: mol_type = other DNA

SEQ ID NO: 41 - protein, 107 aa, synthetic construct
DIVMTQSPKSMSMSVGERVTLSCKASENVGTYVSWYQQKPEQSPKLLIYGASTRESGVPDRFTGSGSGTDFTLTISSVQAEDLAVYYCQNDYSYPFTFGSGTKLEIK

SEQ ID NO: 42 - protein, 11 aa, synthetic construct
KASENVGTYVS

SEQ ID NO: 43 - protein, 7 aa, synthetic construct
GASTRES

SEQ ID NO: 44 - protein, 9 aa, synthetic construct
QNDYSYPFT

SEQ ID NO: 45 - protein, 124 aa, synthetic construct
QVQLQQSGAELVRPGASVTLSCKASGYTFTDYEMHWVKQTPVHGLEWIGVIDPETGGTTYNQKFNDKATLTADKSSSTAYMDLRSLTSEDSAVYYCSRSGYYVSSYESYAMDYWGQGTSVTVSS

SEQ ID NO: 46 - protein, 10 aa, synthetic construct
GYTFTDYEMH

SEQ ID NO: 47 - protein, 10 aa, synthetic construct
VIDPETGGTT

SEQ ID NO: 48 - protein, 15 aa, synthetic construct
SGYYVSSYESYAMDY

SEQ ID NO: 49 - protein, 107 aa, synthetic construct
EIVMTQSPKTMSMSPGERVTLSCKASENVGTYVSWYQQKPGQAPRLLIYGASTRESGVPDRFSGSGSGTDFTLTISSLQPEDFAVYYCQNDYSYPFTFGGGTKLEIK

SEQ ID NO: 50 - protein, 11 aa, synthetic construct
KASENVGTYVS

SEQ ID NO: 51 - protein, 7 aa, synthetic construct
GASTRES

SEQ ID NO: 52 - protein, 9 aa, synthetic construct
QNDYSYPFT

SEQ ID NO: 53 - protein, 124 aa, synthetic construct
QVQLVQSGAEVKKPGASVKVSCKASGYTFTDYEMHWVRQAPGQGLEWMGVIDPETGGTTYNQKFQGRVTLTADTSISTAYMELSRLRSDDTAVYYCSRSGYYVSSYESYAMDYWGQGTTVTVSS

SEQ ID NO: 54 - protein, 10 aa, synthetic construct
GYTFTDYEMH

SEQ ID NO: 55 - protein, 10 aa, synthetic construct
VIDPETGGTT

SEQ ID NO: 56 - protein, 15 aa, synthetic construct
SGYYVSSYESYAMDY

SEQ ID NO: 57 - protein, 107 aa, synthetic construct
EIVMTQSPPTMSMSPGERVTLSCKASENVGTYVSWYQQKPGQAPRLLIYGASTRESGVPARFSGSGSGTDFTLTISSLQPEDFAVYYCQNDYSYPFTFGGGTKLEIK

SEQ ID NO: 58 - protein, 11 aa, synthetic construct
KASENVGTYVS

SEQ ID NO: 59 - protein, 7 aa, synthetic construct
GASTRES

SEQ ID NO: 60 - protein, 9 aa, synthetic construct
QNDYSYPFT

SEQ ID NO: 61 - protein, 124 aa, synthetic construct; identical to SEQ ID NO: 53

SEQ ID NO: 62 - protein, 10 aa, synthetic construct
GYTFTDYEMH

SEQ ID NO: 63 - protein, 10 aa, synthetic construct
VIDPETGGTT

SEQ ID NO: 64 - protein, 15 aa, synthetic construct
SGYYVSSYESYAMDY

SEQ ID NO: 65 - protein, 107 aa, synthetic construct
EIVMTQSPPTLSLSPGERVTLSCRASENVGTYVSWYQQKPGQAPRLLIYGASTRESGIPARFSGSGSGTDFTLTISSLQPEDFAVYYCQNDYSYPFTFGGGTKLEIK

SEQ ID NO: 66 - protein, 11 aa, synthetic construct
RASENVGTYVS

SEQ ID NO: 67 - protein, 7 aa, synthetic construct
GASTRES

SEQ ID NO: 68 - protein, 9 aa, synthetic construct
QNDYSYPFT

SEQ ID NO: 69 - protein, 124 aa, synthetic construct; identical to SEQ ID NO: 53

SEQ ID NO: 70 - protein, 10 aa, synthetic construct
GYTFTDYEMH

SEQ ID NO: 71 - protein, 10 aa, synthetic construct
VIDPETGGTT

SEQ ID NO: 72 - protein, 15 aa, synthetic construct
SGYYVSSYESYAMDY

SEQ ID NO: 73 - protein, 113 aa, synthetic construct
DIVMTQSPSSLTVTAGEKVTMSCKSSQSLLNSGNQKNYLTWYQQKPGQPPKLLIYGASTRESGVPDRFTGSGSGTDFTLTISSVQAEDLAVYYCQNDYSYPFTFGSGTKLEIK

SEQ ID NO: 74 - protein, 17 aa, synthetic construct
KSSQSLLNSGNQKNYLT

SEQ ID NO: 75 - protein, 7 aa, synthetic construct
GASTRES

SEQ ID NO: 76 - protein, 9 aa, synthetic construct
QNDYSYPFT

SEQ ID NO: 77 - protein, 124 aa, synthetic construct
QVQLQQSGAELVRPGASVTLSCKASGYTFTDYEMHWVKQTPVHGLEWIGTIDPETGGTTYNQKFNDKATLTADKSSSTAYMDLRSLTSEDSAVYYCSRSGYYVSSYESYAMDYWGQGTSVTVSS

SEQ ID NO: 78 - protein, 10 aa, synthetic construct
GYTFTDYEMH

SEQ ID NO: 79 - protein, 10 aa, synthetic construct
TIDPETGGTT

SEQ ID NO: 80 - protein, 15 aa, synthetic construct
SGYYVSSYESYAMDY

SEQ ID NO: 81 - protein, 113 aa, synthetic construct
DIVMTQSPDSLAVSLGERATINCKSSQSLLNSGNQKNYLTWYQQKPGQPPKLLIYGASTRESGVPDRFSGSGSGTDFTLTISSLQAEDVAVYYCQNDYSYPFTFGGGTKLEIK

SEQ ID NO: 82 - protein, 17 aa, synthetic construct
KSSQSLLNSGNQKNYLT

SEQ ID NO: 83 - protein, 7 aa, synthetic construct
GASTRES

SEQ ID NO: 84 - protein, 9 aa, synthetic construct
QNDYSYPFT

SEQ ID NO: 85 - protein, 124 aa, synthetic construct
QVQLVQSGAEVKKPGASVKLSCKASGYTFTDYEMHWVRQAPGQGLEWIGTIDPETGGTTYNQKFQGRVTLTADTSISTAYMELSRLRSDDTAVYYCSRSGYYVSSYESYAMDYWGQGTTVTVSS

SEQ ID NO: 86 - protein, 10 aa, synthetic construct
GYTFTDYEMH

SEQ ID NO: 87 - protein, 10 aa, synthetic construct
TIDPETGGTT

SEQ ID NO: 88 - protein, 15 aa, synthetic construct
SGYYVSSYESYAMDY

SEQ ID NO: 89 - protein, 113 aa, synthetic construct
DIVMTQSPDSLAVSLGERVTMNCKSSQSLLNSGNQKNYLTWYQQKPGQPPKLLIYGASTRESGVPDRFSGSGSGTDFTLTISSLQAEDVAVYYCQNDYSYPFTFGGGTKLEIK

SEQ ID NO: 90 - protein, 17 aa, synthetic construct
KSSQSLLNSGNQKNYLT

SEQ ID NO: 91 - protein, 7 aa, synthetic construct
GASTRES

SEQ ID NO: 92 - protein, 9 aa, synthetic construct
QNDYSYPFT

SEQ ID NO: 93 - protein, 124 aa, synthetic construct
QVQLVQSGAEVKKPGASVKVSCKASGYTFTDYEMHWVRQAPGQGLEWMGTIDPETGGTTYAQKFQGRVTLTADTSISTAYMELSRLRSDDTAVYYCSRSGYYVSSYESYAMDYWGQGTTVTVSS

SEQ ID NO: 94 - protein, 10 aa, synthetic construct
GYTFTDYEMH

SEQ ID NO: 95 - protein, 10 aa, synthetic construct
TIDPETGGTT

SEQ ID NO: 96 - protein, 15 aa, synthetic construct
SGYYVSSYESYAMDY

SEQ ID NO: 97 - protein, 113 aa, synthetic construct
DIVMTQSPDSLAVSLGERVTMSCKSSQSLLNSGNQKNYLTWYQQKPGQPPKLLIYGASTRESGVPDRFTGSGSGTDFTLTISSLQAEDVAVYYCQNDYSYPFTFGGGTKLEIK

SEQ ID NO: 98 - protein, 17 aa, synthetic construct
KSSQSLLNSGNQKNYLT

SEQ ID NO: 99 - protein, 7 aa, synthetic construct
GASTRES

SEQ ID NO: 100 - protein, 9 aa, synthetic construct
QNDYSYPFT

SEQ ID NO: 101 - protein, 124 aa, synthetic construct
QVQLVQSGAEVKKPGASVKVSCKASGYTFTDYEMHWVRQAPGQGLEWMGTIDPETGGTTYAQKFQGRVTMTADTSISTAYMELSRLRSDDTAVYYCARSGYYVSSYESYAMDYWGQGTTVTVSS

SEQ ID NO: 102 - protein, 10 aa, synthetic construct
GYTFTDYEMH

SEQ ID NO: 103 - protein, 10 aa, synthetic construct
TIDPETGGTT

SEQ ID NO: 104 - protein, 14 aa, synthetic construct
SGYYVSSYESYAMD

SEQ ID NO: 105 - protein, 113 aa, synthetic construct; identical to SEQ ID NO: 89

SEQ ID NO: 106 - protein, 17 aa, synthetic construct
KSSQSLLNSGNQKNYLT

SEQ ID NO: 107 - protein, 7 aa, synthetic construct
GASTRES

SEQ ID NO: 108 - protein, 9 aa, synthetic construct
QNDYSYPFT

SEQ ID NO: 109 - protein, 124 aa, synthetic construct; identical to SEQ ID NO: 101

SEQ ID NO: 110 - protein, 10 aa, synthetic construct
GYTFTDYEMH

SEQ ID NO: 111 - protein, 10 aa, synthetic construct
TIDPETGGTT

SEQ ID NO: 112 - protein, 14 aa, synthetic construct
SGYYVSSYESYAMD

SEQ ID NO: 113 - protein, 113 aa, synthetic construct
DIVMTQSPPTLSVSPGERVTMSCKSSQSLLNSGNQKNYLTWYQQKPGQAPRLLIYGASTRESGVPDRFSGSGSGTDFTLTISSLQPEDFAVYYCQNDYSYPFTFGGGTKLEIK

SEQ ID NO: 114 - protein, 17 aa, synthetic construct
KSSQSLLNSGNQKNYLT

SEQ ID NO: 115 - protein, 7 aa, synthetic construct
GASTRES

SEQ ID NO: 116 - protein, 9 aa, synthetic construct
QNDYSYPFT

SEQ ID NO: 117 - protein, 124 aa, synthetic construct; identical to SEQ ID NO: 101

SEQ ID NO: 118 - protein, 10 aa, synthetic construct
GYTFTDYEMH

SEQ ID NO: 119 - protein, 10 aa, synthetic construct
TIDPETGGTT

SEQ ID NO: 120 - protein, 14 aa, synthetic construct
SGYYVSSYESYAMD

SEQ ID NO: 121 - protein, 113 aa, synthetic construct
EIVMTQSPPTLSLSPGERVTMSCRSSQSLLNSGNQKNYLTWYQQKPGQAPRLLIYGASTRESGVPARFSGSGSGTDFTLTISSLQPEDFAVYYCQNDYSYPFTFGGGTKLEIK

SEQ ID NO: 122 - protein, 17 aa, synthetic construct
RSSQSLLNSGNQKNYLT

SEQ ID NO: 123 - protein, 7 aa, synthetic construct
GASTRES

SEQ ID NO: 124 - protein, 9 aa, synthetic construct
QNDYSYPFT

SEQ ID NO: 125 - protein, 124 aa, synthetic construct; identical to SEQ ID NO: 101

SEQ ID NO: 126 - protein, 10 aa, synthetic construct
GYTFTDYEMH

SEQ ID NO: 127 - protein, 10 aa, synthetic construct
TIDPETGGTT

SEQ ID NO: 128 - protein, 14 aa, synthetic construct
SGYYVSSYESYAMD

SEQ ID NO: 129 - protein, 107 aa, synthetic construct
DIVMTQSQKFMSTSVGDRVSVTCKASQNVGTNVAWYQQKPGQSPKTLIYSASYRFSGVPDRFTGSGSGTDFTLTINNVQSEDLADYFCQQYNIYPLSFGAGTKLELK

SEQ ID NO: 130 - protein, 11 aa, synthetic construct
KASQNVGTNVA

SEQ ID NO: 131 - protein, 7 aa, synthetic construct
SASYRFS

SEQ ID NO: 132 - protein, 9 aa, synthetic construct
QQYNIYPLS

SEQ ID NO: 133 - protein, 124 aa, synthetic construct
QVQLQQSGAELVRPGASVTLSCKASGYTFTDYEIHWVKQTPVHGLEWIGAIDPETGGTNYNQKFNDKATLTADKSSSTAYMDLRSLTSEDSAVYYCSRSGYYVSNYESYAMDYWGQGTSVTVSS

SEQ ID NO: 134 - protein, 10 aa, synthetic construct
GYTFTDYEIH

SEQ ID NO: 135 - protein, 10 aa, synthetic construct
AIDPETGGTN

SEQ ID NO: 136 - protein, 15 aa, synthetic construct
SGYYVSNYESYAMDY

SEQ ID NO: 137 - protein, 107 aa, synthetic construct
DIQMTQSPSSLSASVGDRVTITCRASQNVGTNVAWYQQKPEKAPKSLIYSASYRFSGVPSRFSGSGSGTDFTLTISSLQPEDFATYYCQQYNIYPLSFGGGTKLELK

SEQ ID NO: 138 - protein, 11 aa, synthetic construct
RASQNVGTNVA

SEQ ID NO: 139 - protein, 7 aa, synthetic construct
SASYRFS

SEQ ID NO: 140 - protein, 9 aa, synthetic construct
QQYNIYPLS

SEQ ID NO: 141 - protein, 124 aa, synthetic construct
QVQLVQSGAEVKKPGASVKVSCKASGYTFTDYEIHWVRQAPGQGLEWIGAIDPETGGTNYNQKFNDRVTLTADKSISTAYMELSRLRSDDTAVYYCSRSGYYVSNYESYAMDYWGQGTTVTVSS

SEQ ID NO: 142 - protein, 10 aa, synthetic construct
GYTFTDYEIH

SEQ ID NO: 143 - protein, 10 aa, synthetic construct
AIDPETGGTN

SEQ ID NO: 144 - protein, 15 aa, synthetic construct
SGYYVSNYESYAMDY

SEQ ID NO: 145 - protein, 107 aa, synthetic construct; identical to SEQ ID NO: 137

SEQ ID NO: 146 - protein, 11 aa, synthetic construct
RASQNVGTNVA

SEQ ID NO: 147 - protein, 7 aa, synthetic construct
SASYRFS

SEQ ID NO: 148 - protein, 9 aa, synthetic construct
QQYNIYPLS

SEQ ID NO: 149 - protein, 124 aa, synthetic construct
QVQLVQSGAEVKKPGASVKVSCKASGYTFTDYEIHWVRQAPGQGLEWIGAIDPETGGTNYNQKFQGRVTLTADTSISTAYMELSRLRSDDTAVYYCSRSGYYVSNYESYAMDYWGQGTTVTVSS

SEQ ID NO: 150 - protein, 10 aa, synthetic construct
GYTFTDYEIH

SEQ ID NO: 151 - protein, 10 aa, synthetic construct
AIDPETGGTN

SEQ ID NO: 152 - protein, 15 aa, synthetic construct
SGYYVSNYESYAMDY

SEQ ID NO: 153 - protein, 107 aa, synthetic construct; identical to SEQ ID NO: 137

SEQ ID NO: 154 - protein, 11 aa, synthetic construct
RASQNVGTNVA

SEQ ID NO: 155 - protein, 7 aa, synthetic construct
SASYRFS

SEQ ID NO: 156 - protein, 9 aa, synthetic construct
QQYNIYPLS

SEQ ID NO: 157 - protein, 124 aa, synthetic construct
QVQLVQSGAEVKKPGASVKVSCKASGYTFTDYEIHWVRQAPGQGLEWMGAIDPETGGTNYAQKFQGRVTMTADTSISTAYMELSRLRSDDTAVYYCSRSGYYVSNYESYAMDYWGQGTTVTVSS

SEQ ID NO: 158 - protein, 10 aa, synthetic construct
GYTFTDYEIH

SEQ ID NO: 159 - protein, 10 aa, synthetic construct
AIDPETGGTN

SEQ ID NO: 160 - protein, 15 aa, synthetic construct
SGYYVSNYESYAMDY

SEQ ID NO: 161 - protein, 107 aa, synthetic construct
DIKITQSPSSMYASLGERVTITCKASQDIKSYLSWYQQKPGSSPRLLIYDTSNLASGVPVRFSGRGSGTSYSLTISRMEAEDAATYYCQQWSSYPFTFGSGTKLEIK

SEQ ID NO: 162 - protein, 11 aa, synthetic construct
KASQDIKSYLS

SEQ ID NO: 163 - protein, 7 aa, synthetic construct
DTSNLAS

SEQ ID NO: 164 - protein, 9 aa, synthetic construct
QQWSSYPFT

SEQ ID NO: 165 - protein, 124 aa, synthetic construct
QLQLQQSGAELVRPGASVTLSCKASGYTFTDYEIHWVKQTPVHGLEWIGAIDPETGGTNYNQKFNDKATLTADKSSSTAYMDLRSLTSEDSAVYYCSRSGYYVSNYESYAMDYWGQGTSVTVSS

SEQ ID NO: 166 - protein, 10 aa, synthetic construct
GYTFTDYEIH

SEQ ID NO: 167 - protein, 10 aa, synthetic construct
AIDPETGGTN

SEQ ID NO: 168 - protein, 15 aa, synthetic construct
SGYYVSNYESYAMDY

SEQ ID NO: 169 - protein, 107 aa, synthetic construct
DIQLTQSPSSLSASVGDRVTITCRASQDIKSYLSWYQQKPGKAPKLLIYDTSNLASGVPSRFSGSGSGTDFTLTISSLQPEDFATYYCQQWSSYPFTFGGGTKLEIK

SEQ ID NO: 170 - protein, 11 aa, synthetic construct
RASQDIKSYLS

SEQ ID NO: 171 - protein, 7 aa, synthetic construct
DTSNLAS

SEQ ID NO: 172 - protein, 9 aa, synthetic construct
QQWSSYPFT

SEQ ID NO: 173 - protein, 124 aa, synthetic construct
QLQLVQSGAEVKKPGASVKVSCKASGYTFTDYEIHWVRQAPGQGLEWIGAIDPETGGTNYNQKFNDRVTLTADTSISTAYMELSRLRSDDTAVYYCSRSGYYVSNYESYAMDYWGQGTTVTVSS

SEQ ID NO: 174 - protein, 10 aa, synthetic construct
GYTFTDYEIH

SEQ ID NO: 175 - protein, 10 aa, synthetic construct
AIDPETGGTN

SEQ ID NO: 176 - protein, 15 aa, synthetic construct
SGYYVSNYESYAMDY

SEQ ID NO: 177 - protein, 107 aa, synthetic construct
DIQITQSPSSMSASVGDRVTITCKASQDIKSYLSWYQQKPGKAPKLLIYDTSNLASGVPSRFSGSGSGTDYTLTISSLQPEDFATYYCQQWSSYPFTFGGGTKLEIK

SEQ ID NO: 178 - protein, 11 aa, synthetic construct
KASQDIKSYLS

SEQ ID NO: 179 - protein, 7 aa, synthetic construct
DTSNLAS

SEQ ID NO: 180 - protein, 9 aa, synthetic construct
QQWSSYPFT

SEQ ID NO: 181 - protein, 124 aa, synthetic construct; identical to SEQ ID NO: 149

SEQ ID NO: 182 - protein, 10 aa, synthetic construct
GYTFTDYEIH

SEQ ID NO: 183 - protein, 10 aa, synthetic construct
AIDPETGGTN

SEQ ID NO: 184 - protein, 15 aa, synthetic construct
SGYYVSNYESYAMDY

SEQ ID NO: 185 - protein, 107 aa, synthetic construct; identical to SEQ ID NO: 177

SEQ ID NO: 186 - protein, 11 aa, synthetic construct
KASQDIKSYLS

SEQ ID NO: 187 - protein, 7 aa, synthetic construct
DTSNLAS

SEQ ID NO: 188 - protein, 9 aa, synthetic construct
QQWSSYPFT

SEQ ID NO: 189 - protein, 124 aa, synthetic construct; identical to SEQ ID NO: 157

SEQ ID NO: 190 - protein, 10 aa, synthetic construct
GYTFTDYEIH

SEQ ID NO: 191 - protein, 10 aa, synthetic construct
AIDPETGGTN

SEQ ID NO: 192 - protein, 15 aa, synthetic construct
SGYYVSNYESYAMDY

SEQ ID NO: 193 - protein, 107 aa, synthetic construct; identical to SEQ ID NO: 169

SEQ ID NO: 194 - protein, 11 aa, synthetic construct
RASQDIKSYLS

SEQ ID NO: 195 - protein, 7 aa, synthetic construct
DTSNLAS

SEQ ID NO: 196 - protein, 9 aa, synthetic construct
QQWSSYPFT

SEQ ID NO: 197 - protein, 124 aa, synthetic construct; identical to SEQ ID NO: 157

SEQ ID NO: 198 - protein, 10 aa, synthetic construct
GYTFTDYEIH

SEQ ID NO: 199 - protein, 10 aa, synthetic construct
AIDPETGGTN

SEQ ID NO: 200 - protein, 15 aa, synthetic construct
SGYYVSNYESYAMDY

SEQ ID NO: 201 - protein, 107 aa, synthetic construct [sequence omitted]

SEQ ID NO: 202 - protein, 330 aa, synthetic construct [sequence omitted]

SEQ ID NO: 203 - protein, 214 aa, synthetic construct
DIVMTQSPKSMSMSVGERVTLSCKASENVGTYVSWYQQKPEQSPKLLIYGASTRESGVPDRFTGSGSGTDFTLTISSVQAEDLAVYYCQNDYSYPFTFGSGTKLEIKRTVAAPSVFIFPPSDEQLKSGTASVVCLLNNFYPREAKVQWKVDNALQSGNSQESVTEQDSKDSTYSLSSTLTLSKADYEKHKVYACEVTHQGLSSPVTKSFNRGEC

SEQ ID NO: 204 - protein, 454 aa, synthetic construct
QVQLQQSGAELVRPGASVTLSCKASGYTFTDYEMHWVKQTPVHGLEWIGVIDPETGGTTYNQKFNDKATLTADKSSSTAYMDLRSLTSEDSAVYYCSRSGYYVSSYESYAMDYWGQGTSVTVSSASTKGPSVFPLAPSSKSTSGGTAALGCLVKDYFPEPVTVSWNSGALTSGVHTFPAVLQSSGLYSLSSVVTVPSSSLGTQTYICNVNHKPSNTKVDKKVEPKSCDKTHTCPPCPAPELLGGPSVFLFPPKPKDTLMISRTPEVTCVVVDVSHEDPEVKFNWYVDGVEVHNAKTKPREEQYNSTYRVVSVLTVLHQDWLNGKEYKCKVSNKALPAPIEKTISKAKGQPREPQVYTLPPSRDELTKNQVSLTCLVKGFYPSDIAVEWESNGQPENNYKTTPPVLDSDGSFFLYSKLTVDKSRWQQGNVFSCSVMHEALHNHYTQKSLSLSPGK

SEQ ID NO: 205 - protein, 214 aa, synthetic construct
EIVMTQSPKTMSMSPGERVTLSCKASENVGTYVSWYQQKPGQAPRLLIYGASTRESGVPDRFSGSGSGTDFTLTISSLQPEDFAVYYCQNDYSYPFTFGGGTKLEIKRTVAAPSVFIFPPSDEQLKSGTASVVCLLNNFYPREAKVQWKVDNALQSGNSQESVTEQDSKDSTYSLSSTLTLSKADYEKHKVYACEVTHQGLSSPVTKSFNRGEC

SEQ ID NO: 206 - protein, 454 aa, synthetic construct
QVQLVQSGAEVKKPGASVKVSCKASGYTFTDYEMHWVRQAPGQGLEWMGVIDPETGGTTYNQKFQGRVTLTADTSISTAYMELSRLRSDDTAVYYCSRSGYYVSSYESYAMDYWGQGTTVTVSSASTKGPSVFPLAPSSKSTSGGTAALGCLVKDYFPEPVTVSWNSGALTSGVHTFPAVLQSSGLYSLSSVVTVPSSSLGTQTYICNVNHKPSNTKVDKKVEPKSCDKTHTCPPCPAPELLGGPSVFLFPPKPKDTLMISRTPEVTCVVVDVSHEDPEVKFNWYVDGVEVHNAKTKPREEQYNSTYRVVSVLTVLHQDWLNGKEYKCKVSNKALPAPIEKTISKAKGQPREPQVYTLPPSRDELTKNQVSLTCLVKGFYPSDIAVEWESNGQPENNYKTTPPVLDSDGSFFLYSKLTVDKSRWQQGNVFSCSVMHEALHNHYTQKSLSLSPGK

SEQ ID NO: 207 - protein, 214 aa, synthetic construct
EIVMTQSPPTMSMSPGERVTLSCKASENVGTYVSWYQQKPGQAPRLLIYGASTRESGVPARFSGSGSGTDFTLTISSLQPEDFAVYYCQNDYSYPFTFGGGTKLEIKRTVAAPSVFIFPPSDEQLKSGTASVVCLLNNFYPREAKVQWKVDNALQSGNSQESVTEQDSKDSTYSLSSTLTLSKADYEKHKVYACEVTHQGLSSPVTKSFNRGEC

SEQ ID NO: 208 - protein, 454 aa, synthetic construct; identical to SEQ ID NO: 206

SEQ ID NO: 209 - protein, 214 aa, synthetic construct
EIVMTQSPPTLSLSPGERVTLSCRASENVGTYVSWYQQKPGQAPRLLIYGASTRESGIPARFSGSGSGTDFTLTISSLQPEDFAVYYCQNDYSYPFTFGGGTKLEIKRTVAAPSVFIFPPSDEQLKSGTASVVCLLNNFYPREAKVQWKVDNALQSGNSQESVTEQDSKDSTYSLSSTLTLSKADYEKHKVYACEVTHQGLSSPVTKSFNRGEC

SEQ ID NO: 210 - protein, 454 aa, synthetic construct; identical to SEQ ID NO: 206

SEQ ID NO: 211 - protein, 220 aa, synthetic construct
DIVMTQSPSSLTVTAGEKVTMSCKSSQSLLNSGNQKNYLTWYQQKPGQPPKLLIYGASTRESGVPDRFTGSGSGTDFTLTISSVQAEDLAVYYCQNDYSYPFTFGSGTKLEIKRTVAAPSVFIFPPSDEQLKSGTASVVCLLNNFYPREAKVQWKVDNALQSGNSQESVTEQDSKDSTYSLSSTLTLSKADYEKHKVYACEVTHQGLSSPVTKSFNRGEC

SEQ ID NO: 212 - protein, 454 aa, synthetic construct
QVQLQQSGAELVRPGASVTLSCKASGYTFTDYEMHWVKQTPVHGLEWIGTIDPETGGTTYNQKFNDKATLTADKSSSTAYMDLRSLTSEDSAVYYCSRSGYYVSSYESYAMDYWGQGTSVTVSSASTKGPSVFPLAPSSKSTSGGTAALGCLVKDYFPEPVTVSWNSGALTSGVHTFPAVLQSSGLYSLSSVVTVPSSSLGTQTYICNVNHKPSNTKVDKKVEPKSCDKTHTCPPCPAPELLGGPSVFLFPPKPKDTLMISRTPEVTCVVVDVSHEDPEVKFNWYVDGVEVHNAKTKPREEQYNSTYRVVSVLTVLHQDWLNGKEYKCKVSNKALPAPIEKTISKAKGQPREPQVYTLPPSRDELTKNQVSLTCLVKGFYPSDIAVEWESNGQPENNYKTTPPVLDSDGSFFLYSKLTVDKSRWQQGNVFSCSVMHEALHNHYTQKSLSLSPGK

SEQ ID NO: 213 - protein, 220 aa, synthetic construct
DIVMTQSPDSLAVSLGERATINCKSSQSLLNSGNQKNYLTWYQQKPGQPPKLLIYGASTRESGVPDRFSGSGSGTDFTLTISSLQAEDVAVYYCQNDYSYPFTFGGGTKLEIKRTVAAPSVFIFPPSDEQLKSGTASVVCLLNNFYPREAKVQWKVDNALQSGNSQESVTEQDSKDSTYSLSSTLTLSKADYEKHKVYACEVTHQGLSSPVTKSFNRGEC

SEQ ID NO: 214 - protein, 454 aa, synthetic construct
QVQLVQSGAEVKKPGASVKLSCKASGYTFTDYEMHWVRQAPGQGLEWIGTIDPETGGTTYNQKFQGRVTLTADTSISTAYMELSRLRSDDTAVYYCSRSGYYVSSYESYAMDYWGQGTTVTVSSASTKGPSVFPLAPSSKSTSGGTAALGCLVKDYFPEPVTVSWNSGALTSGVHTFPAVLQSSGLYSLSSVVTVPSSSLGTQTYICNVNHKPSNTKVDKKVEPKSCDKTHTCPPCPAPELLGGPSVFLFPPKPKDTLMISRTPEVTCVVVDVSHEDPEVKFNWYVDGVEVHNAKTKPREEQYNSTYRVVSVLTVLHQDWLNGKEYKCKVSNKALPAPIEKTISKAKGQPREPQVYTLPPSRDELTKNQVSLTCLVKGFYPSDIAVEWESNGQPENNYKTTPPVLDSDGSFFLYSKLTVDKSRWQQGNVFSCSVMHEALHNHYTQKSLSLSPGK

SEQ ID NO: 215 - protein, 220 aa, synthetic construct
DIVMTQSPDSLAVSLGERVTMNCKSSQSLLNSGNQKNYLTWYQQKPGQPPKLLIYGASTRESGVPDRFSGSGSGTDFTLTISSLQAEDVAVYYCQNDYSYPFTFGGGTKLEIKRTVAAPSVFIFPPSDEQLKSGTASVVCLLNNFYPREAKVQWKVDNALQSGNSQESVTEQDSKDSTYSLSSTLTLSKADYEKHKVYACEVTHQGLSSPVTKSFNRGEC

SEQ ID NO: 216 - protein, 454 aa, synthetic construct
QVQLVQSGAEVKKPGASVKVSCKASGYTFTDYEMHWVRQAPGQGLEWMGTIDPETGGTTYAQKFQGRVTLTADTSISTAYMELSRLRSDDTAVYYCSRSGYYVSSYESYAMDYWGQGTTVTVSSASTKGPSVFPLAPSSKSTSGGTAALGCLVKDYFPEPVTVSWNSGALTSGVHTFPAVLQSSGLYSLSSVVTVPSSSLGTQTYICNVNHKPSNTKVDKKVEPKSCDKTHTCPPCPAPELLGGPSVFLFPPKPKDTLMISRTPEVTCVVVDVSHEDPEVKFNWYVDGVEVHNAKTKPREEQYNSTYRVVSVLTVLHQDWLNGKEYKCKVSNKALPAPIEKTISKAKGQPREPQVYTLPPSRDELTKNQVSLTCLVKGFYPSDIAVEWESNGQPENNYKTTPPVLDSDGSFFLYSKLTVDKSRWQQGNVFSCSVMHEALHNHYTQKSLSLSPGK

SEQ ID NO: 217 - protein, 220 aa, synthetic construct
DIVMTQSPDSLAVSLGERVTMSCKSSQSLLNSGNQKNYLTWYQQKPGQPPKLLIYGASTRESGVPDRFTGSGSGTDFTLTISSLQAEDVAVYYCQNDYSYPFTFGGGTKLEIKRTVAAPSVFIFPPSDEQLKSGTASVVCLLNNFYPREAKVQWKVDNALQSGNSQESVTEQDSKDSTYSLSSTLTLSKADYEKHKVYACEVTHQGLSSPVTKSFNRGEC

SEQ ID NO: 218 - protein, 454 aa, synthetic construct
QVQLVQSGAEVKKPGASVKVSCKASGYTFTDYEMHWVRQAPGQGLEWMGTIDPETGGTTYAQKFQGRVTMTADTSISTAYMELSRLRSDDTAVYYCARSGYYVSSYESYAMDYWGQGTTVTVSSASTKGPSVFPLAPSSKSTSGGTAALGCLVKDYFPEPVTVSWNSGALTSGVHTFPAVLQSSGLYSLSSVVTVPSSSLGTQTYICNVNHKPSNTKVDKKVEPKSCDKTHTCPPCPAPELLGGPSVFLFPPKPKDTLMISRTPEVTCVVVDVSHEDPEVKFNWYVDGVEVHNAKTKPREEQYNSTYRVVSVLTVLHQDWLNGKEYKCKVSNKALPAPIEKTISKAKGQPREPQVYTLPPSRDELTKNQVSLTCLVKGFYPSDIAVEWESNGQPENNYKTTPPVLDSDGSFFLYSKLTVDKSRWQQGNVFSCSVMHEALHNHYTQKSLSLSPGK

SEQ ID NO: 219 - protein, 220 aa, synthetic construct; identical to SEQ ID NO: 215

SEQ ID NO: 220 - protein, 454 aa, synthetic construct; identical to SEQ ID NO: 218

SEQ ID NO: 221 - protein, 220 aa, synthetic construct
DIVMTQSPPTLSVSPGERVTMSCKSSQSLLNSGNQKNYLTWYQQKPGQAPRLLIYGASTRESGVPDRFSGSGSGTDFTLTISSLQPEDFAVYYCQNDYSYPFTFGGGTKLEIKRTVAAPSVFIFPPSDEQLKSGTASVVCLLNNFYPREAKVQWKVDNALQSGNSQESVTEQDSKDSTYSLSSTLTLSKADYEKHKVYACEVTHQGLSSPVTKSFNRGEC

SEQ ID NO: 222 - protein, 454 aa, synthetic construct; identical to SEQ ID NO: 218

SEQ ID NO: 223 - protein, 220 aa, synthetic construct
EIVMTQSPPTLSLSPGERVTMSCRSSQSLLNSGNQKNYLTWYQQKPGQAPRLLIYGASTRESGVPARFSGSGSGTDFTLTISSLQPEDFAVYYCQNDYSYPFTFGGGTKLEIKRTVAAPSVFIFPPSDEQLKSGTASVVCLLNNFYPREAKVQWKVDNALQSGNSQESVTEQDSKDSTYSLSSTLTLSKADYEKHKVYACEVTHQGLSSPVTKSFNRGEC

SEQ ID NO: 224 - protein, 454 aa, synthetic construct; identical to SEQ ID NO: 218

SEQ ID NO: 225 - protein, 214 aa, synthetic construct
DIVMTQSQKFMSTSVGDRVSVTCKASQNVGTNVAWYQQKPGQSPKTLIYSASYRFSGVPDRFTGSGSGTDFTLTINNVQSEDLADYFCQQYNIYPLSFGAGTKLELKRTVAAPSVFIFPPSDEQLKSGTASVVCLLNNFYPREAKVQWKVDNALQSGNSQESVTEQDSKDSTYSLSSTLTLSKADYEKHKVYACEVTHQGLSSPVTKSFNRGEC

SEQ ID NO: 226 - protein, 454 aa, synthetic construct
QVQLQQSGAELVRPGASVTLSCKASGYTFTDYEIHWVKQTPVHGLEWIGAIDPETGGTNYNQKFNDKATLTADKSSSTAYMDLRSLTSEDSAVYYCSRSGYYVSNYESYAMDYWGQGTSVTVSSASTKGPSVFPLAPSSKSTSGGTAALGCLVKDYFPEPVTVSWNSGALTSGVHTFPAVLQSSGLYSLSSVVTVPSSSLGTQTYICNVNHKPSNTKVDKKVEPKSCDKTHTCPPCPAPELLGGPSVFLFPPKPKDTLMISRTPEVTCVVVDVSHEDPEVKFNWYVDGVEVHNAKTKPREEQYNSTYRVVSVLTVLHQDWLNGKEYKCKVSNKALPAPIEKTISKAKGQPREPQVYTLPPSRDELTKNQVSLTCLVKGFYPSDIAVEWESNGQPENNYKTTPPVLDSDGSFFLYSKLTVDKSRWQQGNVFSCSVMHEALHNHYTQKSLSLSPGK

SEQ ID NO: 227 - protein, 214 aa, synthetic construct
DIQMTQSPSSLSASVGDRVTITCRASQNVGTNVAWYQQKPEKAPKSLIYSASYRFSGVPSRFSGSGSGTDFTLTISSLQPEDFATYYCQQYNIYPLSFGGGTKLELKRTVAAPSVFIFPPSDEQLKSGTASVVCLLNNFYPREAKVQWKVDNALQSGNSQESVTEQDSKDSTYSLSSTLTLSKADYEKHKVYACEVTHQGLSSPVTKSFNRGEC

SEQ ID NO: 228 - protein, 454 aa, synthetic construct
QVQLVQSGAEVKKPGASVKVSCKASGYTFTDYEIHWVRQAPGQGLEWIGAIDPETGGTNYNQKFNDRVTLTADKSISTAYMELSRLRSDDTAVYYCSRSGYYVSNYESYAMDYWGQGTTVTVSSASTKGPSVFPLAPSSKSTSGGTAALGCLVKDYFPEPVTVSWNSGALTSGVHTFPAVLQSSGLYSLSSVVTVPSSSLGTQTYICNVNHKPSNTKVDKKVEPKSCDKTHTCPPCPAPELLGGPSVFLFPPKPKDTLMISRTPEVTCVVVDVSHEDPEVKFNWYVDGVEVHNAKTKPREEQYNSTYRVVSVLTVLHQDWLNGKEYKCKVSNKALPAPIEKTISKAKGQPREPQVYTLPPSRDELTKNQVSLTCLVKGFYPSDIAVEWESNGQPENNYKTTPPVLDSDGSFFLYSKLTVDKSRWQQGNVFSCSVMHEALHNHYTQKSLSLSPGK

SEQ ID NO: 229 - protein, 214 aa, synthetic construct; identical to SEQ ID NO: 227

SEQ ID NO: 230 - protein, 454 aa, synthetic construct
QVQLVQSGAEVKKPGASVKVSCKASGYTFTDYEIHWVRQAPGQGLEWIGAIDPETGGTNYNQKFQGRVTLTADTSISTAYMELSRLRSDDTAVYYCSRSGYYVSNYESYAMDYWGQGTTVTVSSASTKGPSVFPLAPSSKSTSGGTAALGCLVKDYFPEPVTVSWNSGALTSGVHTFPAVLQSSGLYSLSSVVTVPSSSLGTQTYICNVNHKPSNTKVDKKVEPKSCDKTHTCPPCPAPELLGGPSVFLFPPKPKDTLMISRTPEVTCVVVDVSHEDPEVKFNWYVDGVEVHNAKTKPREEQYNSTYRVVSVLTVLHQDWLNGKEYKCKVSNKALPAPIEKTISKAKGQPREPQVYTLPPSRDELTKNQVSLTCLVKGFYPSDIAVEWESNGQPENNYKTTPPVLDSDGSFFLYSKLTVDKSRWQQGNVFSCSVMHEALHNHYTQKSLSLSPGK

SEQ ID NO: 231 - protein, 214 aa, synthetic construct; identical to SEQ ID NO: 227

SEQ ID NO: 232 - protein, 454 aa, synthetic construct
QVQLVQSGAEVKKPGASVKVSCKASGYTFTDYEIHWVRQAPGQGLEWMGAIDPETGGTNYAQKFQGRVTMTADTSISTAYMELSRLRSDDTAVYYCSRSGYYVSNYESYAMDYWGQGTTVTVSSASTKGPSVFPLAPSSKSTSGGTAALGCLVKDYFPEPVTVSWNSGALTSGVHTFPAVLQSSGLYSLSSVVTVPSSSLGTQTYICNVNHKPSNTKVDKKVEPKSCDKTHTCPPCPAPELLGGPSVFLFPPKPKDTLMISRTPEVTCVVVDVSHEDPEVKFNWYVDGVEVHNAKTKPREEQYNSTYRVVSVLTVLHQDWLNGKEYKCKVSNKALPAPIEKTISKAKGQPREPQVYTLPPSRDELTKNQVSLTCLVKGFYPSDIAVEWESNGQPENNYKTTPPVLDSDGSFFLYSKLTVDKSRWQQGNVFSCSVMHEALHNHYTQKSLSLSPGK

SEQ ID NO: 233 - protein, 214 aa, synthetic construct
DIKITQSPSSMYASLGERVTITCKASQDIKSYLSWYQQKPGSSPRLLIYDTSNLASGVPVRFSGRGSGTSYSLTISRMEAEDAATYYCQQWSSYPFTFGSGTKLEIKRTVAAPSVFIFPPSDEQLKSGTASVVCLLNNFYPREAKVQWKVDNALQSGNSQESVTEQDSKDSTYSLSSTLTLSKADYEKHKVYACEVTHQGLSSPVTKSFNRGEC

SEQ ID NO: 234 - protein, 454 aa, synthetic construct
QLQLQQSGAELVRPGASVTLSCKASGYTFTDYEIHWVKQTPVHGLEWIGAIDPETGGTNYNQKFNDKATLTADKSSSTAYMDLRSLTSEDSAVYYCSRSGYYVSNYESYAMDYWGQGTSVTVSSASTKGPSVFPLAPSSKSTSGGTAALGCLVKDYFPEPVTVSWNSGALTSGVHTFPAVLQSSGLYSLSSVVTVPSSSLGTQTYICNVNHKPSNTKVDKKVEPKSCDKTHTCPPCPAPELLGGPSVFLFPPKPKDTLMISRTPEVTCVVVDVSHEDPEVKFNWYVDGVEVHNAKTKPREEQYNSTYRVVSVLTVLHQDWLNGKEYKCKVSNKALPAPIEKTISKAKGQPREPQVYTLPPSRDELTKNQVSLTCLVKGFYPSDIAVEWESNGQPENNYKTTPPVLDSDGSFFLYSKLTVDKSRWQQGNVFSCSVMHEALHNHYTQKSLSLSPGK

SEQ ID NO: 235 - protein, 214 aa, synthetic construct
DIQLTQSPSSLSASVGDRVTITCRASQDIKSYLSWYQQKPGKAPKLLIYDTSNLASGVPSRFSGSGSGTDFTLTISSLQPEDFATYYCQQWSSYPFTFGGGTKLEIKRTVAAPSVFIFPPSDEQLKSGTASVVCLLNNFYPREAKVQWKVDNALQSGNSQESVTEQDSKDSTYSLSSTLTLSKADYEKHKVYACEVTHQGLSSPVTKSFNRGEC

SEQ ID NO: 236 - protein, 454 aa, synthetic construct
QLQLVQSGAEVKKPGASVKVSCKASGYTFTDYEIHWVRQAPGQGLEWIGAIDPETGGTNYNQKFNDRVTLTADTSISTAYMELSRLRSDDTAVYYCSRSGYYVSNYESYAMDYWGQGTTVTVSSASTKGPSVFPLAPSSKSTSGGTAALGCLVKDYFPEPVTVSWNSGALTSGVHTFPAVLQSSGLYSLSSVVTVPSSSLGTQTYICNVNHKPSNTKVDKKVEPKSCDKTHTCPPCPAPELLGGPSVFLFPPKPKDTLMISRTPEVTCVVVDVSHEDPEVKFNWYVDGVEVHNAKTKPREEQYNSTYRVVSVLTVLHQDWLNGKEYKCKVSNKALPAPIEKTISKAKGQPREPQVYTLPPSRDELTKNQVSLTCLVKGFYPSDIAVEWESNGQPENNYKTTPPVLDSDGSFFLYSKLTVDKSRWQQGNVFSCSVMHEALHNHYTQKSLSLSPGK

SEQ ID NO: 237 - protein, 214 aa, synthetic construct
DIQITQSPSSMSASVGDRVTITCKASQDIKSYLSWYQQKPGKAPKLLIYDTSNLASGVPSRFSGSGSGTDYTLTISSLQPEDFATYYCQQWSSYPFTFGGGTKLEIKRTVAAPSVFIFPPSDEQLKSGTASVVCLLNNFYPREAKVQWKVDNALQSGNSQESVTEQDSKDSTYSLSSTLTLSKADYEKHKVYACEVTHQGLSSPVTKSFNRGEC

SEQ ID NO: 238 - protein, 454 aa, synthetic construct; identical to SEQ ID NO: 230

SEQ ID NO: 239 - protein, 214 aa, synthetic construct; identical to SEQ ID NO: 237

SEQ ID NO: 240 - protein, 454 aa, synthetic construct; identical to SEQ ID NO: 232

SEQ ID NO: 241 - protein, 214 aa, synthetic construct; identical to SEQ ID NO: 235

SEQ ID NO: 242 - protein, 454 aa, synthetic construct; identical to SEQ ID NO: 232